European Patent Application EP 4 134 376 A1, published February 15, 2023. Title: Process of Manufacture. Applicant: Annexin Pharmaceuticals AB. The sequence listing filed with the application follows.

SEQUENCE LISTING (2 sequences)

SEQ ID NO: 1 - protein, 320 aa, Homo sapiens
  Amino acid sequence of human Annexin A5
MAQVLRGTVTDFPGFDERADAETLRKAMKGLGTDEESILTLLTSRSNAQRQEISAAFKTLFGRDLLDDLKSELTGKFEKLIVALMKPSRLYDAYELKHALKGAGTNEKVLTEIIASRTPEELRAIKQVYEEEYGSSLEDDVVGDTSGYYQRMLVVLLQANRDPDAGIDEAQVEQDAQALFQAGELKWGTDEEKFITIFGTRSVSHLRKVFDKYMTISGFQIEETIDRETSGNLEQLLLAVVKSIRSIPAYLAETLYYAMKGAGTDDHTLIRVMVSRSEIDLFNIRKEFRKNFATSLYSMIKGDTSGDYKKALLLLCGEDD

SEQ ID NO: 2 - protein, 362 aa, Homo sapiens
  Amino acid sequence of human TIM-1
MHPQVVILSLILHLADSVAGSVKVGGEAGPSVTLPCHYSGAVTSMCWRGSCSLFTCQNGIVWTNGTHVTYRKDTRYKLLGDLSRRDVSLTIENTAVSDSGVYCCRVEHRGWFNDMKITVSLEIVPPKVTTTPIVTTVPTVTTVRTSTTVPTTTTVPMTTVPTTTVPTTMSIPTTTTVLTTMTVSTTTSVPTTTSIPTTTSVPVTTTVSTFVPPMPLPRQNHEPVATSPSSPQPAETHPTTLQGAIRREPTSSPLYSYTTDGNDTVTESSDGLWNNQTQLFLEHSLLTANTTKGIYAGVCISVLVLLALLGVIIAKKYFFKKEVQQLSVSFSSLQIKALQNAVEKEVQAEDNIYIENSLYATD